European Patent Application EP 4 265 644 A1, published October 25, 2023. Title: BISPECIFIC ANTIBODY FOR SPECIFICALLY NEUTRALIZING TGF-beta SIGNAL OF HELPER T CELL, AND PHARMACEUTICAL COMPOSITION AND USE THEREOF. Applicant: Shenzhen Majory Biotechnology Co.,Ltd. The sequence listing filed with the application follows.

SEQUENCE LISTING (83 sequences)

SEQ ID NO: 1 - protein, 122 aa, Artificial Sequence
QVQLQQSGPEVVKPGASVKMSCKASGYTFTSYVIHWVRQKPGQGLDWIGYINPYNDGTDYDEKFKGKATLTSDTSTSTAYMELSSLRSEDTAVYYCAREKDNYATGAWFAYWGQGTLVTVSS

SEQ ID NO: 2 - protein, 112 aa, Artificial Sequence
DIVMTQSPDSLAVSLGERVTMNCKSSQSLLYSTNQKNYLAWYQQKPGQSPKLLIYWASTRESGVPDRFSGSGSGTDFTLTISSVQAEDVAVYYCQQYYSYRTFGGGTKLEIK

SEQ ID NO: 3 - protein, 123 aa, Artificial Sequence
EVQLVESGGGVVQPGRSLRLSCAASGFTFSSYGMHWVRQAPGKELEWVAVISYDGSIKYYADSVKGRFTISRDNSKNTLYLQMNSLRAEDTAVYYCARTGEYSGYDTDPQYSWGQGTTVTVSS

SEQ ID NO: 4 - protein, 123 aa, Artificial Sequence
EVQLVESGGGVVQPGRSLRLSCAASGFTFSSYGMHWVRQAPGKELEWVAVISYDGSIKYYADSVKGRFTISRDNSKNTLYLQMNSLRAEDTAVYYCARTGEYSGYDTSGVELWGQGTTVTVSS

SEQ ID NO: 5 - protein, 123 aa, Artificial Sequence
EVQLVESGGGVVQPGRSLRLSCAASGFTFSSYGMHWVRQAPGKELEWVAVISYDGSIKYYADSVKGRFTISRDNSKNTLYLQMNSLRAEDTAVYYCARTGFYSGYDTPASPDWGQGTTVTVSS

SEQ ID NO: 6 - protein, 107 aa, Artificial Sequence
EIVLTQSPSSLSASVGDRVTITCRASQGIGDDLGWYQQKPGKAPILLIYGTSTLQSGVPSRFSGSGSGTDFTLTINSLQPEDFATYYCLQDSNYPLTFGGGTRLEIK

SEQ ID NO: 7 - protein, 15 aa, Artificial Sequence
GGGGSGGGGSGGGGS

SEQ ID NO: 8 - protein, 5 aa, Artificial Sequence
GGGGS

SEQ ID NO: 9 - protein, 107 aa, Artificial Sequence
GTVAAPSVFIFPPSDEQLKSGTASVVCLLNNFYPREAKVQWKVDNALQSGNSQESVTEQDSKDSTYSLSSTLTLSKADYEKHKVYACEVTHQGLSSPVTKSFNRGEC

SEQ ID NO: 10 - protein, 100 aa, Artificial Sequence
ASTKGPSVFPLAPCSRSTSESTAALGCLVKDYFPEPVTVSWNSGALTSGVHTFPAVLQSSGLYSLSSVVTVPSSSLGTKTYTCNVDHKPSNTKVDKRVES

SEQ ID NO: 11 - protein, 18 aa, Artificial Sequence
KYGPPCPPCPAPEFLGGP

SEQ ID NO: 12 - protein, 209 aa, Artificial Sequence
SVFLFPPKPKDTLMISRTPEVTCVVVDVSQEDPEVQFNWYVDGVEVHNAKTKPREEQFNSTYRVVSVLTVLHQDWLNGKEYKCKVSNKGLPSSIEKTISKAKGQPREPQVYTLPPSQEEMTKNQVSLTCLVKGFYPSDIAVEWESNGQPENNYKTTPPVLDSDGSFFLYSRLTVDKSRWQEGNVFSCSVMHEALHNHYTQKSLSLSLGK

SEQ ID NO: 13 - protein, 219 aa, Artificial Sequence
DIVMTQSPDSLAVSLGERVTMNCKSSQSLLYSTNQKNYLAWYQQKPGQSPKLLIYWASTRESGVPDRFSGSGSGTDFTLTISSVQAEDVAVYYCQQYYSYRTFGGGTKLEIKGTVAAPSVFIFPPSDEQLKSGTASVVCLLNNFYPREAKVQWKVDNALQSGNSQESVTEQDSKDSTYSLSSTLTLSKADYEKHKVYACEVTHQGLSSPVTKSFNRGEC

SEQ ID NO: 14 - protein, 709 aa, Artificial Sequence
QVQLQQSGPEVVKPGASVKMSCKASGYTFTSYVIHWVRQKPGQGLDWIGYINPYNDGTDYDEKFKGKATLTSDTSTSTAYMELSSLRSEDTAVYYCAREKDNYATGAWFAYWGQGTLVTVSSASTKGPSVFPLAPCSRSTSESTAALGCLVKDYFPEPVTVSWNSGALTSGVHTFPAVLQSSGLYSLSSVVTVPSSSLGTKTYTCNVDHKPSNTKVDKRVESKYGPPCPPCPAPEFLGGPSVFLFPPKPKDTLMISRTPEVTCVVVDVSQEDPEVQFNWYVDGVEVHNAKTKPREEQFNSTYRVVSVLTVLHQDWLNGKEYKCKVSNKGLPSSIEKTISKAKGQPREPQVYTLPPSQEEMTKNQVSLTCLVKGFYPSDIAVEWESNGQPENNYKTTPPVLDSDGSFFLYSRLTVDKSRWQEGNVFSCSVMHEALHNHYTQKSLSLSLGKGGGGSGGGGSGGGGSEVQLVESGGGVVQPGRSLRLSCAASGFTFSSYGMHWVRQAPGKELEWVAVISYDGSIKYYADSVKGRFTISRDNSKNTLYLQMNSLRAEDTAVYYCARTGEYSGYDTDPQYSWGQGTTVTVSSGGGGSGGGGSGGGGSEIVLTQSPSSLSASVGDRVTITCRASQGIGDDLGWYQQKPGKAPILLIYGTSTLQSGVPSRFSGSGSGTDFTLTINSLQPEDFATYYCLQDSNYPLTFGGGTRLEIK

SEQ ID NO: 15 - protein, 479 aa, Artificial Sequence
DIVMTQSPDSLAVSLGERVTMNCKSSQSLLYSTNQKNYLAWYQQKPGQSPKLLIYWASTRESGVPDRFSGSGSGTDFTLTISSVQAEDVAVYYCQQYYSYRTFGGGTKLEIKGTVAAPSVFIFPPSDEQLKSGTASVVCLLNNFYPREAKVQWKVDNALQSGNSQESVTEQDSKDSTYSLSSTLTLSKADYEKHKVYACEVTHQGLSSPVTKSFNRGECGGGGSGGGGSGGGGSEVQLVESGGGVVQPGRSLRLSCAASGFTFSSYGMHWVRQAPGKELEWVAVISYDGSIKYYADSVKGRFTISRDNSKNTLYLQMNSLRAEDTAVYYCARTGEYSGYDTDPQYSWGQGTTVTVSSGGGGSGGGGSGGGGSEIVLTQSPSSLSASVGDRVTITCRASQGIGDDLGWYQQKPGKAPILLIYGTSTLQSGVPSRFSGSGSGTDFTLTINSLQPEDFATYYCLQDSNYPLTFGGGTRLEIK

SEQ ID NO: 16 - protein, 449 aa, Artificial Sequence
QVQLQQSGPEVVKPGASVKMSCKASGYTFTSYVIHWVRQKPGQGLDWIGYINPYNDGTDYDEKFKGKATLTSDTSTSTAYMELSSLRSEDTAVYYCAREKDNYATGAWFAYWGQGTLVTVSSASTKGPSVFPLAPCSRSTSESTAALGCLVKDYFPEPVTVSWNSGALTSGVHTFPAVLQSSGLYSLSSVVTVPSSSLGTKTYTCNVDHKPSNTKVDKRVESKYGPPCPPCPAPEFLGGPSVFLFPPKPKDTLMISRTPEVTCVVVDVSQEDPEVQFNWYVDGVEVHNAKTKPREEQFNSTYRVVSVLTVLHQDWLNGKEYKCKVSNKGLPSSIEKTISKAKGQPREPQVYTLPPSQEEMTKNQVSLTCLVKGFYPSDIAVEWESNGQPENNYKTTPPVLDSDGSFFLYSRLTVDKSRWQEGNVFSCSVMHEALHNHYTQKSLSLSLGK

SEQ ID NO: 17 - protein, 219 aa, Artificial Sequence; identical to SEQ ID NO: 13

SEQ ID NO: 18 - protein, 709 aa, Artificial Sequence
EVQLVESGGGVVQPGRSLRLSCAASGFTFSSYGMHWVRQAPGKELEWVAVISYDGSIKYYADSVKGRFTISRDNSKNTLYLQMNSLRAEDTAVYYCARTGEYSGYDTDPQYSWGQGTTVTVSSGGGGSGGGGSGGGGSEIVLTQSPSSLSASVGDRVTITCRASQGIGDDLGWYQQKPGKAPILLIYGTSTLQSGVPSRFSGSGSGTDFTLTINSLQPEDFATYYCLQDSNYPLTFGGGTRLEIKGGGGSGGGGSGGGGSQVQLQQSGPEVVKPGASVKMSCKASGYTFTSYVIHWVRQKPGQGLDWIGYINPYNDGTDYDEKFKGKATLTSDTSTSTAYMELSSLRSEDTAVYYCAREKDNYATGAWFAYWGQGTLVTVSSASTKGPSVFPLAPCSRSTSESTAALGCLVKDYFPEPVTVSWNSGALTSGVHTFPAVLQSSGLYSLSSVVTVPSSSLGTKTYTCNVDHKPSNTKVDKRVESKYGPPCPPCPAPEFLGGPSVFLFPPKPKDTLMISRTPEVTCVVVDVSQEDPEVQFNWYVDGVEVHNAKTKPREEQFNSTYRVVSVLTVLHQDWLNGKEYKCKVSNKGLPSSIEKTISKAKGQPREPQVYTLPPSQEEMTKNQVSLTCLVKGFYPSDIAVEWESNGQPENNYKTTPPVLDSDGSFFLYSRLTVDKSRWQEGNVFSCSVMHEALHNHYTQKSLSLSLGK

SEQ ID NO: 19 - protein, 479 aa, Artificial Sequence
EVQLVESGGGVVQPGRSLRLSCAASGFTFSSYGMHWVRQAPGKELEWVAVISYDGSIKYYADSVKGRFTISRDNSKNTLYLQMNSLRAEDTAVYYCARTGEYSGYDTDPQYSWGQGTTVTVSSGGGGSGGGGSGGGGSEIVLTQSPSSLSASVGDRVTITCRASQGIGDDLGWYQQKPGKAPILLIYGTSTLQSGVPSRFSGSGSGTDFTLTINSLQPEDFATYYCLQDSNYPLTFGGGTRLEIKGGGGSGGGGSGGGGSDIVMTQSPDSLAVSLGERVTMNCKSSQSLLYSTNQKNYLAWYQQKPGQSPKLLIYWASTRESGVPDRFSGSGSGTDFTLTISSVQAEDVAVYYCQQYYSYRTFGGGTKLEIKGTVAAPSVFIFPPSDEQLKSGTASVVCLLNNFYPREAKVQWKVDNALQSGNSQESVTEQDSKDSTYSLSSTLTLSKADYEKHKVYACEVTHQGLSSPVTKSFNRGEC

SEQ ID NO: 20 - protein, 449 aa, Artificial Sequence; identical to SEQ ID NO: 16

SEQ ID NO: 21 - protein, 331 aa, Artificial Sequence
EIVLTQSPSSLSASVGDRVTITCRASQGIGDDLGWYQQKPGKAPILLIYGTSTLQSGVPSRFSGSGSGTDFTLTINSLQPEDFATYYCLQDSNYPLTFGGGTRLEIKGGGGSDIVMTQSPDSLAVSLGERVTMNCKSSQSLLYSTNQKNYLAWYQQKPGQSPKLLIYWASTRESGVPDRFSGSGSGTDFTLTISSVQAEDVAVYYCQQYYSYRTFGGGTKLEIKGTVAAPSVFIFPPSDEQLKSGTASVVCLLNNFYPREAKVQWKVDNALQSGNSQESVTEQDSKDSTYSLSSTLTLSKADYEKHKVYACEVTHQGLSSPVTKSFNRGEC

SEQ ID NO: 22 - protein, 577 aa, Artificial Sequence
EVQLVESGGGVVQPGRSLRLSCAASGFTFSSYGMHWVRQAPGKELEWVAVISYDGSIKYYADSVKGRFTISRDNSKNTLYLQMNSLRAEDTAVYYCARTGEYSGYDTDPQYSWGQGTTVTVSSGGGGSQVQLQQSGPEVVKPGASVKMSCKASGYTFTSYVIHWVRQKPGQGLDWIGYINPYNDGTDYDEKFKGKATLTSDTSTSTAYMELSSLRSEDTAVYYCAREKDNYATGAWFAYWGQGTLVTVSSASTKGPSVFPLAPCSRSTSESTAALGCLVKDYFPEPVTVSWNSGALTSGVHTFPAVLQSSGLYSLSSVVTVPSSSLGTKTYTCNVDHKPSNTKVDKRVESKYGPPCPPCPAPEFLGGPSVFLFPPKPKDTLMISRTPEVTCVVVDVSQEDPEVQFNWYVDGVEVHNAKTKPREEQFNSTYRVVSVLTVLHQDWLNGKEYKCKVSNKGLPSSIEKTISKAKGQPREPQVYTLPPSQEEMTKNQVSLTCLVKGFYPSDIAVEWESNGQPENNYKTTPPVLDSDGSFFLYSRLTVDKSRWQEGNVFSCSVMHEALHNHYTQKSLSLSLGK

SEQ ID NO: 23 - protein, 219 aa, Artificial Sequence; identical to SEQ ID NO: 13

SEQ ID NO: 24 - protein, 449 aa, Artificial Sequence
QVQLQQSGPEVVKPGASVKMSCKASGYTFTSYVIHWVRQKPGQGLDWIGYINPYNDGTDYDEKFKGKATLTSDTSTSTAYMELSSLRSEDTAVYYCAREKDNYATGAWFAYWGQGTLVTVSSASTKGPSVFPLAPCSRSTSESTAALGCLVKDYFPEPVTVSWNSGALTSGVHTFPAVLQSSGLYSLSSVVTVPSSSLGTKTYTCNVDHKPSNTKVDKRVESKYGPPCPPCPAPEFLGGPSVFLFPPKPKDTLMISRTPEVTCVVVDVSQEDPEVQFNWYVDGVEVHNAKTKPREEQFNSTYRVVSVLTVLHQDWLNGKEYKCKVSNKGLPSSIEKTISKAKGQPREPQVYTLPPCQEEMTKNQVSLWCLVKGFYPSDIAVEWESNGQPENNYKTTPPVLDSDGSFFLYSALTVDKSRWQEGNVFSCSVMHEALHNHYTQKSLSLSLGK

SEQ ID NO: 25 - protein, 698 aa, Artificial Sequence
EVQLVESGGGVVQPGRSLRLSCAASGFTFSSYGMHWVRQAPGKELEWVAVISYDGSIKYYADSVKGRFTISRDNSKNTLYLQMNSLRAEDTAVYYCARTGEYSGYDTDPQYSWGQGTTVTVSGGSGTVAAPSVFIFPPSDEQLKSGTASVVCLLNNFYPREAKVQWKVDNALQSGNSQESVTEQDSKDSTYSLSSTLTLSKADYEKHKVYACEVTHQGLSSPVTKSFNRGECSGGGGSEVQLVESGGGVVQPGRSLRLSCAASGFTFSSYGMHWVRQAPGKELEWVAVISYDGSIKYYADSVKGRFTISRDNSKNTLYLQMNSLRAEDTAVYYCARTGEYSGYDTDPQYSWGQGTTVTVSGGSGTVAAPSVFIFPPSDEQLKSGTASVVCLLNNFYPREAKVQWKVDNALQSGNSQESVTEQDSKDSTYSLSSTLTLSKADYEKHKVYACEVTHQGLSSPVTKSFNRGECSKYGPPCPPCPAPEFLGGPSVFLFPPKPKDTLMISRTPEVTCVVVDVSQEDPEVQFNWYVDGVEVHNAKTKPREEQFNSTYRVVSVLTVLHQDWLNGKEYKCKVSNKGLPSSIEKTISKAKGQPREPQVCTLPPSQEEMTKNQVSLSCAVKGFYPSDIAVEWESNGQPENNYKTTPPVLDSDGSFKLVSRLTVDKSRWQEGNVFSCSVMHEALHNHYTQKSLSLSLGK

SEQ ID NO: 26 - protein, 210 aa, Artificial Sequence
EIVLTQSPSSLSASVGDRVTITCRSSQGIGDDLGWYQQKPGKAPILLIYGTSTLQSGVPSRFSGSGSGTDFTLTINSLQPEDFATYYCLQDSNYPLTFGGGTRLEIKGSSASTKGPSVFPLAPCSRSTSESTAALGCLVKDYFPEPVTVSWNSGALTSGVHTFPAVLQSSGLYSLSSVVTVPSSSLGTKTYTCNVDHKPSNTKVDKRVES

SEQ ID NO: 27 - protein, 210 aa, Artificial Sequence; identical to SEQ ID NO: 26

SEQ ID NO: 28 - protein, 460 aa, Artificial Sequence
EVQLVESGGGVVQPGRSLRLSCAASGFTFSSYGMHWVRQAPGKELEWVAVISYDGSIKYYADSVKGRFTISRDNSKNTLYLQMNSLRAEDTAVYYCARTGEYSGYDTDPQYSWGQGTTVTVSGGSGTVAAPSVFIFPPSDEQLKSGTASVVCLLNNFYPREAKVQWKVDNALQSGNSQESVTEQDSKDSTYSLSSTLTLSKADYEKHKVYACEVTHQGLSSPVTKSFNRGECSKYGPPCPPCPAPEFLGGPSVFLFPPKPKDTLMISRTPEVTCVVVDVSQEDPEVQFNWYVDGVEVHNAKTKPREEQFNSTYRVVSVLTVLHQDWLNGKEYKCKVSNKGLPSSIEKTISKAKGQPREPQVYTLPPCQEEMTKNQVSLWCLVKGFYPSDIAVEWESNGQPENNYKTTPPVLDSDGSFFLYSALTVDKSRWQEGNVFSCSVMHEALHNHYTQKSLSLSLGK

SEQ ID NO: 29 - protein, 687 aa, Artificial Sequence
QVQLQQSGPEVVKPGASVKMSCKASGYTFTSYVIHWVRQKPGQGLDWIGYINPYNDGTDYDEKFKGKATLTSDTSTSTAYMELSSLRSEDTAVYYCAREKDNYATGAWFAYWGQGTLVTVSSASTKGPSVFPLAPCSRSTSESTAALGCLVKDYFPEPVTVSWNSGALTSGVHTFPAVLQSSGLYSLSSVVTVPSSSLGTKTYTCNVDHKPSNTKVDKRVESGGGGSEVQLVESGGGVVQPGRSLRLSCAASGFTFSSYGMHWVRQAPGKELEWVAVISYDGSIKYYADSVKGRFTISRDNSKNTLYLQMNSLRAEDTAVYYCARTGEYSGYDTDPQYSWGQGTTVTVSGGSGTVAAPSVFIFPPSDEQLKSGTASVVCLLNNFYPREAKVQWKVDNALQSGNSQESVTEQDSKDSTYSLSSTLTLSKADYEKHKVYACEVTHQGLSSPVTKSFNRGECSKYGPPCPPCPAPEFLGGPSVFLFPPKPKDTLMISRTPEVTCVVVDVSQEDPEVQFNWYVDGVEVHNAKTKPREEQFNSTYRVVSVLTVLHQDWLNGKEYKCKVSNKGLPSSIEKTISKAKGQPREPQVCTLPPSQEEMTKNQVSLSCAVKGFYPSDIAVEWESNGQPENNYKTTPPVLDSDGSFKLVSRLTVDKSRWQEGNVFSCSVMHEALHNHYTQKSLSLSLGK

SEQ ID NO: 30 - protein, 219 aa, Artificial Sequence; identical to SEQ ID NO: 13

SEQ ID NO: 31 - protein, 219 aa, Artificial Sequence; identical to SEQ ID NO: 13

SEQ ID NO: 32 - protein, 210 aa, Artificial Sequence; identical to SEQ ID NO: 26

SEQ ID NO: 33 - protein, 687 aa, Artificial Sequence
QVQLQQSGPEVVKPGASVKMSCKASGYTFTSYVIHWVRQKPGQGLDWIGYINPYNDGTDYDEKFKGKATLTSDTSTSTAYMELSSLRSEDTAVYYCAREKDNYATGAWFAYWGQGTLVTVSSASTKGPSVFPLAPCSRSTSESTAALGCLVKDYFPEPVTVSWNSGALTSGVHTFPAVLQSSGLYSLSSVVTVPSSSLGTKTYTCNVDHKPSNTKVDKRVESGGGGSEVQLVESGGGVVQPGRSLRLSCAASGFTFSSYGMHWVRQAPGKELEWVAVISYDGSIKYYADSVKGRFTISRDNSKNTLYLQMNSLRAEDTAVYYCARTGEYSGYDTDPQYSWGQGTTVTVSGGSGTVAAPSVFIFPPSDEQLKSGTASVVCLLNNFYPREAKVQWKVDNALQSGNSQESVTEQDSKDSTYSLSSTLTLSKADYEKHKVYACEVTHQGLSSPVTKSFNRGECSKYGPPCPPCPAPEFLGGPSVFLFPPKPKDTLMISRTPEVTCVVVDVSQEDPEVQFNWYVDGVEVHNAKTKPREEQFNSTYRVVSVLTVLHQDWLNGKEYKCKVSNKGLPSSIEKTISKAKGQPREPQVYTLPPSQEEMTKNQVSLTCLVKGFYPSDIAVEWESNGQPENNYKTTPPVLDSDGSFFLYSRLTVDKSRWQEGNVFSCSVMHEALHNHYTQKSLSLSLGK

SEQ ID NO: 34 - protein, 219 aa, Artificial Sequence; identical to SEQ ID NO: 13

SEQ ID NO: 35 - protein, 210 aa, Artificial Sequence; identical to SEQ ID NO: 26

SEQ ID NO: 36 - protein, 696 aa, Artificial Sequence
QVQLQQSGPEVVKPGASVKMSCKASGYTFTSYVIHWVRQKPGQGLDWIGYINPYNDGTDYDEKFKGKATLTSDTSTSTAYMELSSLRSEDTAVYYCAREKDNYATGAWFAYWGQGTLVTVSSASTKGPSVFPLAPCSRSTSESTAALGCLVKDYFPEPVTVSWNSGALTSGVHTFPAVLQSSGLYSLSSVVTVPSSSLGTKTYTCNVDHKPSNTKVDKRVESKYGPPCPPCPAPEFLGGPSVFLFPPKPKDTLMISRTPEVTCVVVDVSQEDPEVQFNWYVDGVEVHNAKTKPREEQFNSTYRVVSVLTVLHQDWLNGKEYKCKVSNKGLPSSIEKTISKAKGQPREPQVYTLPPSQEEMTKNQVSLTCLVKGFYPSDIAVEWESNGQPENNYKTTPPVLDSDGSFFLYSRLTVDKSRWQEGNVFSCSVMHEALHNHYTQKSLSLSLGKGGGGSGGGGSGGGGSEVQLVESGGGVVQPGRSLRLSCAASGFTFSSYGMHWVRQAPGKELEWVAVISYDGSIKYYADSVKGRFTISRDNSKNTLYLQMNSLRAEDTAVYYCARTGEYSGYDTDPQYSWGQGTTVTVSGGSGTVAAPSVFIFPPSDEQLKSGTASVVCLLNNFYPREAKVQWKVDNALQSGNSQESVTEQDSKDSTYSLSSTLTLSKADYEKHKVYACEVTHQGLSSPVTKSFNRGEC

SEQ ID NO: 37 - protein, 219 aa, Artificial Sequence; identical to SEQ ID NO: 13

SEQ ID NO: 38 - protein, 577 aa, Artificial Sequence
QVQLQQSGPEVVKPGASVKMSCKASGYTFTSYVIHWVRQKPGQGLDWIGYINPYNDGTDYDEKFKGKATLTSDTSTSTAYMELSSLRSEDTAVYYCAREKDNYATGAWFAYWGQGTLVTVSSASTKGPSVFPLAPCSRSTSESTAALGCLVKDYFPEPVTVSWNSGALTSGVHTFPAVLQSSGLYSLSSVVTVPSSSLGTKTYTCNVDHKPSNTKVDKRVESKYGPPCPPCPAPEFLGGPSVFLFPPKPKDTLMISRTPEVTCVVVDVSQEDPEVQFNWYVDGVEVHNAKTKPREEQFNSTYRVVSVLTVLHQDWLNGKEYKCKVSNKGLPSSIEKTISKAKGQPREPQVYTLPPCQEEMTKNQVSLWCLVKGFYPSDIAVEWESNGQPENNYKTTPPVLDSDGSFFLYSALTVDKSRWQEGNVFSCSVMHEALHNHYTQKSLSLSLGKGGGGSEVQLVESGGGVVQPGRSLRLSCAASGFTFSSYGMHWVRQAPGKELEWVAVISYDGSIKYYADSVKGRFTISRDNSKNTLYLQMNSLRAEDTAVYYCARTGEYSGYDTDPQYSWGQGTTVTVSS

SEQ ID NO: 39 - protein, 561 aa, Artificial Sequence
QVQLQQSGPEVVKPGASVKMSCKASGYTFTSYVIHWVRQKPGQGLDWIGYINPYNDGTDYDEKFKGKATLTSDTSTSTAYMELSSLRSEDTAVYYCAREKDNYATGAWFAYWGQGTLVTVSSASTKGPSVFPLAPCSRSTSESTAALGCLVKDYFPEPVTVSWNSGALTSGVHTFPAVLQSSGLYSLSSVVTVPSSSLGTKTYTCNVDHKPSNTKVDKRVESKYGPPCPPCPAPEFLGGPSVFLFPPKPKDTLMISRTPEVTCVVVDVSQEDPEVQFNWYVDGVEVHNAKTKPREEQFNSTYRVVSVLTVLHQDWLNGKEYKCKVSNKGLPSSIEKTISKAKGQPREPQVCTLPPSQEEMTKNQVSLSCAVKGFYPSDIAVEWESNGQPENNYKTTPPVLDSDGSFKLVSRLTVDKSRWQEGNVFSCSVMHEALHNHYTQKSLSLSLGKGGGGSEIVLTQSPSSLSASVGDRVTITCRASQGIGDDLGWYQQKPGKAPILLIYGTSTLQSGVPSRFSGSGSGTDFTLTINSLQPEDFATYYCLQDSNYPLTFGGGTRLEIK

SEQ ID NO: 40 - protein, 219 aa, Artificial Sequence; identical to SEQ ID NO: 13

SEQ ID NO: 41 - protein, 449 aa, Artificial Sequence; identical to SEQ ID NO: 24

SEQ ID NO: 42 - protein, 471 aa, Artificial Sequence
EVQLVESGGGVVQPGRSLRLSCAASGFTFSSYGMHWVRQAPGKELEWVAVISYDGSIKYYADSVKGRFTISRDNSKNTLYLQMNSLRAEDTAVYYCARTGEYSGYDTDPQYSWGQGTTVTVSSGGGGSGGGGSGGGGSEIVLTQSPSSLSASVGDRVTITCRASQGIGDDLGWYQQKPGKAPILLIYGTSTLQSGVPSRFSGSGSGTDFTLTINSLQPEDFATYYCLQDSNYPLTFGGGTRLEIKYGPPCPPCPAPEFLGGPSVFLFPPKPKDTLMISRTPEVTCVVVDVSQEDPEVQFNWYVDGVEVHNAKTKPREEQFNSTYRVVSVLTVLHQDWLNGKEYKCKVSNKGLPSSIEKTISKAKGQPREPQVCTLPPSQEEMTKNQVSLSCAVKGFYPSDIAVEWESNGQPENNYKTTPPVLDSDGSFKLVSRLTVDKSRWQEGNVFSCSVMHEALHNHYTQKSLSLSLGK

SEQ ID NO: 43 - protein, 219 aa, Artificial Sequence; identical to SEQ ID NO: 13

SEQ ID NO: 44 - protein, 449 aa, Artificial Sequence; identical to SEQ ID NO: 24

SEQ ID NO: 45 - protein, 460 aa, Artificial Sequence
EVQLVESGGGVVQPGRSLRLSCAASGFTFSSYGMHWVRQAPGKELEWVAVISYDGSIKYYADSVKGRFTISRDNSKNTLYLQMNSLRAEDTAVYYCARTGEYSGYDTDPQYSWGQGTTVTVSGGSGTVAAPSVFIFPPSDEQLKSGTASVVCLLNNFYPREAKVQWKVDNALQSGNSQESVTEQDSKDSTYSLSSTLTLSKADYEKHKVYACEVTHQGLSSPVTKSFNRGECSKYGPPCPPCPAPEFLGGPSVFLFPPKPKDTLMISRTPEVTCVVVDVSQEDPEVQFNWYVDGVEVHNAKTKPREEQFNSTYRVVSVLTVLHQDWLNGKEYKCKVSNKGLPSSIEKTISKAKGQPREPQVCTLPPSQEEMTKNQVSLSCAVKGFYPSDIAVEWESNGQPENNYKTTPPVLDSDGSFKLVSRLTVDKSRWQEGNVFSCSVMHEALHNHYTQKSLSLSLGK

SEQ ID NO: 46 - protein, 210 aa, Artificial Sequence; identical to SEQ ID NO: 26

SEQ ID NO: 47 - protein, 475 aa, Artificial Sequence
EVQLVESGGGVVQPGRSLRLSCAASGFTFSSYGMHWVRQAPGKELEWVAVISYDGSIKYYADSVKGRFTISRDNSKNTLYLQMNSLRAEDTAVYYCARTGEYSGYDTDPQYSWGQGTTVTVSSGGGGSGGGGSGGGGSEIVLTQSPSSLSASVGDRVTITCRASQGIGDDLGWYQQKPGKAPILLIYGTSTLQSGVPSRFSGSGSGTDFTLTINSLQPEDFATYYCLQDSNYPLTFGGGTRLEIKSGSKYGPPCPPCPAPEFLGGPSVFLFPPKPKDTLMISRTPEVTCVVVDVSQEDPEVQFNWYVDGVEVHNAKTKPREEQFNSTYRVVSVLTVLHQDWLNGKEYKCKVSNKGLPSSIEKTISKAKGQPREPQVYTLPPSQEEMTKNQVSLTCLVKGFYPSDIAVEWESNGQPENNYKTTPPVLDSDGSFFLYSRLTVDKSRWQEGNVFSCSVMHEALHNHYTQKSLSLSLGK

SEQ ID NO: 48 - protein, 475 aa, Artificial Sequence
EVQLVESGGGLVQPGGSLRLSCAASGYTFTNYGMNWVRQAPGKGLEWVGWINTYTGEPTYAADFKRRFTFSLDTSKSTAYLQMNSLRAEDTAVYYCAKYPHYYGSSHWYFDVWGQGTLVTVSSGGGGSGGGGSGGGGSDIQMTQSPSSLSASVGDRVTITCSASQDISNYLNWYQQKPGKAPKVLIYFTSSLHSGVPSRFSGSGSGTDFTLTISSLQPEDFATYYCQQYSTVPWTFGQGTKVEIKSGSKYGPPCPPCPAPEFLGGPSVFLFPPKPKDTLMISRTPEVTCVVVDVSQEDPEVQFNWYVDGVEVHNAKTKPREEQFNSTYRVVSVLTVLHQDWLNGKEYKCKVSNKGLPSSIEKTISKAKGQPREPQVYTLPPSQEEMTKNQVSLTCLVKGFYPSDIAVEWESNGQPENNYKTTPPVLDSDGSFFLYSRLTVDKSRWQEGNVFSCSVMHEALHNHYTQKSLSLSLGK

SEQ ID NO: 49 - protein, 371 aa, Artificial Sequence
KKVVLGKKGDTVELTCTASQKKSIQFHWKNSNQIKILGNQGSFLTKGPSKLNDRADSRRSLWDQGNFPLIIKNLKIEDSDTYICEVEDQKEEVQLLVFGLTANSDTHLLQGQSLTLTLESPPGSSPSVQCRSPRGKNIQGGKTLSVSQLELQDSGTWTCTVLQNQKKVEFKIDIVVLAFQKASSIVYKKEGEQVEFSFPLAFTVEKLTGSGELWWQAERASSSKSWITFDLKNKEVSVKRVTQDPKLQMGKKLPLHLTLPQALPQYAGSGNLTLALEAKTGKLHQEVNLVVMRATQLQKNLTCEVWGPTSPKLMLSLKLENKEAKVSKREKAVWVLNPEAGMWQCLLSDSGQVLLESNIKVLPTWHHHHHH

SEQ ID NO: 50 - DNA, 1113 bp, Artificial Sequence
aagaaagtggtgctgggcaaaaaaggggatacagtggaactgacctgtacagcttcccagaagaagagcatacaattccactggaaaaactccaaccagataaagattctgggaaatcagggctccttcttaactaaaggtccatccaagctgaatgatcgcgctgactcaagaagaagcctttgggaccaaggaaactttcccctgatcatcaagaatcttaagatagaagactcagatacttacatctgtgaagtggaggaccagaaggaggaggtgcaattgctagtgttcggattgactgccaactctgacacccacctgcttcaggggcagagcctgaccctgaccttggagagcccccctggtagtagcccctcagtgcaatgtaggagtccaaggggtaaaaacatacagggggggaagaccctctccgtgtctcagctggagctccaggatagtggcacctggacatgcactgtcttgcagaaccagaagaaggtggagttcaaaatagacatcgtggtgctagctttccagaaggcctccagcatagtctataagaaagagggggaacaggtggagttctccttcccactcgcctttacagttgaaaagctgacgggcagtggcgagctgtggtggcaggcggagagggcttcctcctccaagtcttggatcacctttgacctgaagaacaaggaagtgtctgtaaaacgggttacccaggaccctaagctccagatgggcaagaagctcccgctccacctcaccctgccccaggccttgcctcagtatgctggctctggaaacctcaccctggcccttgaagcgaaaacaggaaagttgcatcaggaagtgaacctggtggtgatgagagccactcagctccagaaaaatttgacctgtgaggtgtggggacccacctcccctaagctgatgctgagtttgaaactggagaacaaggaggcaaaggtctcgaagcgggagaaggcggtgtgggtgctgaaccctgaggcggggatgtggcagtgtctgctgagtgactcgggacaggtcctgctggaatccaacatcaaggttctgcccacatggcatcatcatcatcatcat

SEQ ID NO: 51 - protein, 118 aa, Artificial Sequence
ALDTNYCFSSTEKNCCVRQLYIDFRKDLGWKWIHEPKGYHANFCLGPCPYIWSLDTQYSKVLALYNQHNPGASAAPCCVPQALEPLPIVYYVGRKPKVEQLSNMIVRSCKCSHHHHHH

SEQ ID NO: 52 - DNA, 354 bp, Artificial Sequence
gccctggataccaactattgcttcagctccacagagaagaactgctgtgtgcggcagctgtacattgactttaggaaggacctgggttggaagtggatccacgagcccaagggctaccatgccaacttctgcctcgggccctgcccctacatttggagcctggacacgcagtacagcaaggtcctggccctgtacaaccagcataacccgggcgcctcggcggcgccgtgctgcgtgccgcaggcgctggagccgctgcccatcgtgtactacgtgggccgcaagcccaaggtggagcagctgtccaacatgatcgtgcgctcctgcaagtgcagccatcatcatcatcatcat

SEQ ID NO: 53 - protein, 10 aa, Artificial Sequence
GYTFTSYVIH

SEQ ID NO: 54 - protein, 17 aa, Artificial Sequence
YINPYNDGTDYDEKFKG

SEQ ID NO: 55 - protein, 12 aa, Artificial Sequence
EKDNYATGAWFA

SEQ ID NO: 56 - protein, 17 aa, Artificial Sequence
KSSQSLLYSTNQKNYLA

SEQ ID NO: 57 - protein, 7 aa, Artificial Sequence
WASTRES

SEQ ID NO: 58 - protein, 8 aa, Artificial Sequence
QQYYSYRT

SEQ ID NO: 59 - protein, 5 aa, Artificial Sequence
SYGMH

SEQ ID NO: 60 - protein, 17 aa, Artificial Sequence
VISYDGSIKYYADSVKG

SEQ ID NO: 61 - protein, 14 aa, Artificial Sequence
TGEYSGYDTDPQYS

SEQ ID NO: 62 - protein, 14 aa, Artificial Sequence
TGEYSGYDTSGVEL

SEQ ID NO: 63 - protein, 14 aa, Artificial Sequence
TGFYSGYDTPASPD

SEQ ID NO: 64 - protein, 14 aa, Artificial Sequence
TGXYSGYDTXXXXX

SEQ ID NO: 65 - protein, 11 aa, Artificial Sequence
RSSQGIGDDLG

SEQ ID NO: 66 - protein, 7 aa, Artificial Sequence
GTSTLQS

SEQ ID NO: 67 - protein, 9 aa, Artificial Sequence
LQDSNYPLT

SEQ ID NO: 68 - protein, 475 aa, Artificial Sequence; identical to SEQ ID NO: 47

SEQ ID NO: 69 - protein, 475 aa, Artificial Sequence; identical to SEQ ID NO: 48

SEQ ID NO: 70 - protein, 118 aa, Artificial Sequence; identical to SEQ ID NO: 51

SEQ ID NO: 71 - DNA, 354 bp, Artificial Sequence; identical to SEQ ID NO: 52

SEQ ID NO: 72 - protein, 371 aa, Artificial Sequence; identical to SEQ ID NO: 49

SEQ ID NO: 73 - DNA, 1113 bp, Artificial Sequence; identical to SEQ ID NO: 50

SEQ ID NO: 74 - protein, 370 aa, Artificial Sequence
TIPPHVQKSVNNDMIVTDNNGAVKFPQLCKFCDVRFSTCDNQKSCMSNCSITSICEKPQEVCVAVWRKNDENITLETVCHDPKLPYHDFILEDAASPKCIMKEKKKPGETFFMCSCSSDECNDNIIFSEEYNTSNPDLVPRGSDKTHTCPPCPAPELLGGPSVFLFPPKPKDTLMISRTPEVTCVVVDVSHEDPEVKFNWYVDGVEVHNAKTKPREEQYNSTYRVVSVLTVLHQDWLNGKEYKCKVSNKALPAPIEKTISKAKGQPREPQVYTLPPSREEMTKNQVSLTCLVKGFYPSDIAVEWESNGQPENNYKTTPPVLDSDGSFFLYSKLTVDKSRWQQGNVFSCSVMHEALHNHYTQKSLSLSPGK

SEQ ID NO: 75 - DNA, 1110 bp, Artificial Sequence
acgatcccaccgcacgttcagaagtcggttaataacgacatgatagtcactgacaacaacggtgcagtcaagtttccacaactgtgtaaattttgtgatgtgagattttccacctgtgacaaccagaaatcctgcatgagcaactgcagcatcacctccatctgtgagaagccacaggaagtctgtgtggctgtatggagaaagaatgacgagaacataacactagagacagtttgccatgaccccaagctcccctaccatgactttattctggaagatgctgcttctccaaagtgcattatgaaggaaaaaaaaaagcctggtgagactttcttcatgtgttcctgtagctctgatgagtgcaatgacaacatcatcttctcagaagaatataacaccagcaatcctgacctggtgccgaggggaagcgacaaaactcacacatgcccaccgtgcccagcacctgaactcctggggggaccgtcagtcttcctcttccccccaaaacccaaggacaccctcatgatctcccggacccctgaggtcacatgcgtggtggtggacgtgagccacgaagaccctgaggtcaagttcaactggtacgtggacggcgtggaggtgcataatgccaagacaaagccgcgggaggagcagtacaacagcacgtaccgtgtggtcagcgtcctcaccgtcctgcaccaggactggctgaatggcaaggagtacaagtgcaaggtctccaacaaagccctcccagcccccatcgagaaaaccatctccaaagccaaagggcagccccgagaaccacaggtgtacaccctgcccccatcccgggaggagatgaccaagaaccaggtcagcctgacctgcctggtcaaaggcttctatcccagcgacatcgccgtggagtgggagagcaatgggcagccggagaacaactacaagaccacgcctcccgtgctggactccgacggctccttcttcctctacagcaagctcaccgtggacaagagcaggtggcagcaggggaacgtcttctcatgctccgtgatgcatgaggctctgcacaaccactacacgcagaagagcctctccctgtctccgggtaaa

SEQ ID NO: 76 - protein, 122 aa, Artificial Sequence; identical to SEQ ID NO: 1

SEQ ID NO: 77 - DNA, 366 bp, Artificial Sequence
caggtgcaactgcaacagtccggacccgaagtcgtgaaaccaggagcttccgtgaagatgagctgcaaagcatccggatacaccttcaccagctacgtgatccactgggtgaggcagaaacctggccagggcctggactggatcggctacatcaacccttacaacgacggaaccgactacgacgagaaattcaaaggcaaagctaccctgaccagcgacaccagcacctccactgcttacatggagctgtccagcctgaggtccgaagacaccgctgtgtactactgcgctagggagaaggacaactacgctaccggcgcttggttcgcctactggggccagggaaccctggtgaccgtgtccagc

SEQ ID NO: 78 - protein, 112 aa, Artificial Sequence; identical to SEQ ID NO: 2

SEQ ID NO: 79 - DNA, 336 bp, Artificial Sequence
gacatcgtgatgacccagtcccctgactccctggctgtgtccctgggcgaacgggtcaccatgaactgcaaatcttcccagtccctgctgtactccaccaaccagaagaactacctggcttggtaccagcagaaacctggccagtcccccaaactgctcatctactgggcttccaccagggaaagcggcgtgcctgacagattctccggaagcggcagcggaaccgacttcaccctgaccatctccagcgtgcaggctgaagacgtggctgtctactactgccagcagtactacagctacaggaccttcggcggaggcaccaagctggagatcaag

SEQ ID NO: 80 - protein, 123 aa, Artificial Sequence; identical to SEQ ID NO: 3

SEQ ID NO: 81 - DNA, 369 bp, Artificial Sequence
gaggtccagctggtggagtctgggggaggcgtggtccagcctgggaggtccctgagactctcctgtgcagcctctggattcaccttcagtagctatggcatgcactgggtccgccaggctccaggcaaggagctggagtgggtggcagttatatcatatgatggaagtattaaatactatgcagactccgtgaagggccgattcaccatctccagagacaattccaagaacacgctgtatctgcaaatgaacagcctgagagctgaggacacggctgtgtattactgtgcgcgaactggtgaatatagtggctacgatacggacccccagtactcctgggggcaagggaccacggtcaccgtctcctca

SEQ ID NO: 82 - protein, 107 aa, Artificial Sequence
EIVLTQSPSSLSASVGDRVTITCRSSQGIGDDLGWYQQKPGKAPILLIYGTSTLQSGVPSRFSGSGSGTDFTLTINSLQPEDFATYYCLQDSNYPLTFGGGTRLEIK

SEQ ID NO: 83 - DNA, 321 bp, Artificial Sequence
gaaattgtgctgactcagtctccatcctccctgtctgcatctgtaggagacagagtcaccatcacttgccggtcaagtcagggcattggagatgatttgggctggtatcagcagaagccagggaaagcccctatcctcctgatctatggtacatccactttacaaagtggggtcccgtcaaggttcagcggcagtggatctggcacagatttcactctcaccatcaacagcctgcagcctgaagattttgcaacttattactgtctacaagattccaattacccgctcactttcggcggagggacacgactggagattaaa